European Patent Specification EP 3 332 765 B1, published June 5, 2024. Title: An Improving Agent for Skin Sugging or Aging comprising an Adipose Stem Cells-attracting Agent. Applicant: Shiseido Company, Limited. The sequence listing filed with the application follows.

SEQUENCE LISTING (4 sequences)

SEQ ID NO: 1 - DNA, 20 bp, Artificial Sequence
  Primer
agcaggcaaacctggtgaac

SEQ ID NO: 2 - DNA, 20 bp, Artificial Sequence
  Primer
aacctctctcgcctcttgct

SEQ ID NO: 3 - DNA, 20 bp, Artificial Sequence
  Primer
acggtaacgcaggtgtccta

SEQ ID NO: 4 - DNA, 20 bp, Artificial Sequence
  Primer
ccgctttcacggtctgtatt